European Patent Specification EP 3 790 571 B1, published August 14, 2024. Title: OCA-B Peptide Conjugates and Methods of Treatment. Applicant: University of Utah Research Foundation. The sequence listing filed with the application follows.

SEQUENCE LISTING (36 sequences)

SEQ ID NO: 1 - protein, 14 aa, Artificial Sequence
  Synthetic construct
ARPYQGVRVKEPVK

SEQ ID NO: 2 - protein, 11 aa, Artificial Sequence
  Synthetic construct
VKELLRRKRGH

SEQ ID NO: 3 - protein, 23 aa, Artificial Sequence
  Synthetic construct
ARPYQGVRVKEPVKELLRRKRGH

SEQ ID NO: 4 - protein, 12 aa, Artificial Sequence
  Synthetic construct
GRKKRRQRRRGY

SEQ ID NO: 5 - protein, 256 aa, Mus musculus
MLWQKSTAPEQAPAPPRPYQGVRVKEPVKELLRRKRGHTSVGAAGPPTAVVLPHQPLATYSTVGPSCLDMEVSASTVTEEGTLCAGWLSQPAPATLQPLAPWTPYTEYVSHEAVSCPYSTDMYVQPVCPSYTVVGPSSVLTYASPPLITNVTPRSTATPAVGPQLEGPEHQAPLTYFPWPQPLSTLPTSSLQYQPPAPTLSGPQFVQLPISIPEPVLQDMDDPRRAISSLTIDKLLLEEEESNTYELNHTLSVEGF

SEQ ID NO: 6 - protein, 16 aa, Artificial Sequence
  Penetratin
RQIKIWFQNRRMKWKK

SEQ ID NO: 7 - protein, 256 aa, Homo sapiens
MLWQKPTAPEQAPAPARPYQGVRVKEPVKELLRRKRGHASSGAAPAPTAVVLPHQPLATYTTVGPSCLDMEGSVSAVTEEAALCAGWLSQPTPATLQPLAPWTPYTEYVPHEAVSCPYSADMYVQPVCPSYTVVGPSSVLTYASPPLITNVTTRSSATPAVGPPLEGPEHQAPLTYFPWPQPLSTLPTSTLQYQPPAPALPGPQFVQLPISIPEPVLQDMEDPRRAASSLTIDKLLLEEEDSDAYALNHTLSVEGF

SEQ ID NO: 8 - protein, 13 aa, Artificial Sequence
  Synthetic construct
GRKKRRQRRRPPQ

SEQ ID NO: 9 - protein, 26 aa, Artificial Sequence
  Synthetic construct
EPVKEPVKKELLRRKRGHSVGAAGPP

SEQ ID NO: 10 - protein, 26 aa, Artificial Sequence
  Synthetic construct
VKELLRRKRGHGSGGRKKRRQRRRGY

SEQ ID NO: 11 - protein, 11 aa, Artificial Sequence
  Synthetic construct
AKELLRRKRGH

SEQ ID NO: 12 - protein, 11 aa, Artificial Sequence
  Synthetic construct
VAELLRRKRGH

SEQ ID NO: 13 - protein, 11 aa, Artificial Sequence
  Synthetic construct
VKALLRRKRGH

SEQ ID NO: 14 - protein, 11 aa, Artificial Sequence
  Synthetic construct
VKEALRRKRGH

SEQ ID NO: 15 - protein, 11 aa, Artificial Sequence
  Synthetic construct
VKELARRKRGH

SEQ ID NO: 16 - protein, 11 aa, Artificial Sequence
  Synthetic construct
VKELLARKRGH

SEQ ID NO: 17 - protein, 11 aa, Artificial Sequence
  Synthetic construct
VKELLRAKRGH

SEQ ID NO: 18 - protein, 11 aa, Artificial Sequence
  Synthetic construct
VKELLRRARGH

SEQ ID NO: 19 - protein, 11 aa, Artificial Sequence
  Synthetic construct
VKELLRRKAGH

SEQ ID NO: 20 - protein, 11 aa, Artificial Sequence
  Synthetic construct
VKELLRRKRAH

SEQ ID NO: 21 - protein, 11 aa, Artificial Sequence
  Synthetic construct
VKELLRRKRGA

SEQ ID NO: 22 - protein, 11 aa, Artificial Sequence
  Synthetic construct
CKELLRRKRGH

SEQ ID NO: 23 - protein, 11 aa, Artificial Sequence
  Synthetic construct
VCELLRRKRGH

SEQ ID NO: 24 - protein, 11 aa, Artificial Sequence
  Synthetic construct
VKCLLRRKRGH

SEQ ID NO: 25 - protein, 11 aa, Artificial Sequence
  Synthetic construct
VKECLRRKRGH

SEQ ID NO: 26 - protein, 11 aa, Artificial Sequence
  Synthetic construct
VKELCRRKRGH

SEQ ID NO: 27 - protein, 11 aa, Artificial Sequence
  Synthetic construct
VKELLCRKRGH

SEQ ID NO: 28 - protein, 11 aa, Artificial Sequence
  Synthetic construct
VKELLRCKRGH

SEQ ID NO: 29 - protein, 11 aa, Artificial Sequence
  Synthetic construct
VKELLRRCRGH

SEQ ID NO: 30 - protein, 11 aa, Artificial Sequence
  Synthetic construct
VKELLRRKCGH

SEQ ID NO: 31 - protein, 11 aa, Artificial Sequence
  Synthetic construct
VKELLRRKRCH

SEQ ID NO: 32 - protein, 11 aa, Artificial Sequence
  Synthetic construct
VKELLRRKRGC

SEQ ID NO: 33 - protein, 20 aa, Artificial Sequence
  Synthetic construct
LSSPSALNSPGIEGLSRRRK

SEQ ID NO: 34 - protein, 20 aa, Artificial Sequence
  Synthetic construct
AALLSSLNELGERQLVHWKW

SEQ ID NO: 35 - protein, 21 aa, Artificial Sequence
  Synthetic construct
MEVGWYRSPFSRVVHLYRNGK

SEQ ID NO: 36 - protein, 9 aa, Artificial Sequence
  Synthetic construct
CLLRRKRGC